European Patent Specification EP 3 639 821 B1, published August 28, 2024. Title: Carcinogenesis inhibitor. Applicant: National Cancer Center Nippon Zoki Pharmaceutical Co., Ltd. The sequence listing filed with the application follows.

SEQUENCE LISTING (6 sequences)

SEQ ID NO: 1 - DNA, 20 bp, Artificial Sequence
  Primer
  Inventor: MUTOH, Michihiro; KUROKAWA, Yurie; FUJII, Gen; MIYAMOTO, Shingo
gcccgcgcccagacaggata

SEQ ID NO: 2 - DNA, 16 bp, Artificial Sequence
  Primer
gcggcggcggagagga

SEQ ID NO: 3 - DNA, 21 bp, Artificial Sequence
  Primer
atggctgccactcgatatgaa

SEQ ID NO: 4 - DNA, 22 bp, Artificial Sequence
  Primer
tgctcctccattaggaactctc

SEQ ID NO: 5 - DNA, 20 bp, Artificial Sequence
  Primer
tgactgccgagaagttgtgc

SEQ ID NO: 6 - DNA, 19 bp, Artificial Sequence
  Primer
ctcatccgcctctggcatt